European Patent Specification EP 3 349 811 B1, published April 12, 2023. Title: Peptid zur Beschichtung von Oberflächen. Applicant: Universitaet Leipzig. The sequence listing filed with the application follows.

SEQUENCE LISTING (8 sequences)

SEQ ID NO: 1 - protein, 7 aa, Artificial Sequence
  Heparin-bindende Sequenz
FHRRIKA

SEQ ID NO: 2 - protein, 8 aa, Artificial Sequence
  Hauptkette, abgeleitet von einem Protein aus Mytilus edulis
  MISC_FEATURE (2)..(2): Xaa ist Amino-PEG-Säure, vorzugsweise Amino-PEG3-Säure (-HN-CH2-CH2-O-CH2-CH2-O-CH2-CH2-O-CH2-CH2-CO-)
  MISC_FEATURE (3)..(3): Xaa ist L-3,4-Dihydroxyphenylalanin (DOPA)
  MISC_FEATURE (5)..(5): Xaa ist L-3,4-Dihydroxyphenylalanin (DOPA)
  MISC_FEATURE (6)..(6): Xaa ist Amino-PEG-Säure, vorzugsweise Amino-PEG3-Säure (-HN-CH2-CH2-O-CH2-CH2-O-CH2-CH2-O-CH2-CH2-CO-)
  MISC_FEATURE (7)..(7): Xaa ist L-Propargylglycin
  MOD_RES (8)..(8): AMIDATION, bAla
CXXKXXXX

SEQ ID NO: 3 - protein, 10 aa, Artificial Sequence
  bio-MP
  MOD_RES (1)..(1): Acp
  MISC_FEATURE (1)..(1): N-terminal biotinyliert
  MOD_RES (2)..(2): Acp
  MISC_FEATURE (4)..(4): Xaa ist Amino-PEG3-Säure (-HN-CH2-CH2-O-CH2-CH2-O-CH2-CH2-O-CH2-CH2-CO-)
  MISC_FEATURE (5)..(5): Xaa ist L-3,4-Dihydroxyphenylalanin
  MISC_FEATURE (7)..(7): Xaa ist L-3,4-Dihydroxyphenylalanin
  MISC_FEATURE (8)..(8): Xaa ist Amino-PEG3-Säure (-HN-CH2-CH2-O-CH2-CH2-O-CH2-CH2-O-CH2-CH2-CO-)
  MISC_FEATURE (9)..(9): Xaa ist Propargylglycin
  MOD_RES (10)..(10): AMIDATION, bAla
XXCXXKXXXX

SEQ ID NO: 4 - protein, 12 aa, Artificial Sequence
  bio-(+)mefp-1
  MOD_RES (1)..(1): Acp
  MISC_FEATURE (1)..(1): N-terminal biotinyliert
  MOD_RES (2)..(2): Acp
  MOD_RES (5)..(5): 4Hyp
  MISC_FEATURE (7)..(7): Xaa ist L-3,4-Dihydroxyphenylalanin
  MOD_RES (8)..(8): 4Hyp
  MOD_RES (9)..(9): 4Hyp
  MISC_FEATURE (11)..(11): Xaa ist L-3,4-Dihydroxyphenylalanin
  MOD_RES (12)..(12): AMIDATION
XXAKXSXXXTXK

SEQ ID NO: 5 - protein, 12 aa, Artificial Sequence
  bio-(-)mefp-1
  MOD_RES (1)..(1): Acp
  MISC_FEATURE (1)..(1): N-terminal biotinyliert
  MOD_RES (2)..(2): Acp
  MOD_RES (5)..(5): 4Hyp
  MOD_RES (8)..(8): 4Hyp
  MOD_RES (9)..(9): 4Hyp
  MOD_RES (12)..(12): AMIDATION
XXAKPSYPPTYK

SEQ ID NO: 6 - protein, 8 aa, Artificial Sequence
  MP-Ahx
  MOD_RES (2)..(2): Acp
  MISC_FEATURE (3)..(3): Xaa ist L-3,4-Dihydroxyphenylalanin
  MISC_FEATURE (5)..(5): Xaa ist L-3,4-Dihydroxyphenylalanin
  MOD_RES (6)..(6): Acp
  MISC_FEATURE (7)..(7): Xaa ist Propargylglycin
  MOD_RES (8)..(8): AMIDATION, bAla
CXXKXXXX

SEQ ID NO: 7 - protein, 8 aa, Artificial Sequence
  N3-HBP
  MISC_FEATURE (1)..(1): Xaa ist Azidolysin (N3-Lysin)
  MOD_RES (8)..(8): AMIDATION
XFHRRIKA

SEQ ID NO: 8 - protein, 8 aa, Artificial Sequence
  MP
  MISC_FEATURE (2)..(2): Xaa ist Amino-PEG3-Säure (-HN-CH2-CH2-O-CH2-CH2-O-CH2-CH2-O-CH2-CH2-CO-)
  MISC_FEATURE (3)..(3): Xaa ist L-3,4-Dihydroxyphenylalanin
  MISC_FEATURE (5)..(5): Xaa ist L-3,4-Dihydroxyphenylalanin
  MISC_FEATURE (6)..(6): Xaa ist Amino-PEG3-Säure (-HN-CH2-CH2-O-CH2-CH2-O-CH2-CH2-O-CH2-CH2-CO-)
  MISC_FEATURE (7)..(7): Xaa ist Propargylglycin
  MOD_RES (8)..(8): AMIDATION, bAla
CXXKXXXX